European Patent Specification EP 3 473 274 B1, published December 18, 2024. Title: A novel platform for antibody drug conjugate using a bispecific antibody. Applicant: SEOUL NATIONAL UNIVERSITY R&DB FOUNDATION. The sequence listing filed with the application follows.

SEQUENCE LISTING (10 sequences)

SEQ ID NO: 1 - DNA, 357 bp, Artificial Sequence
  heavy chain of anti-cotinine scFv
gaggtgcagctggtggagagcgggggcggcctggtgcagcctggaggaagcctgcgactgtcctgtgcagcttctggacacctgcggagaagggactggatgaactgggtgcggcaggcaccaggaaaaggcctggagtgggtcgcagccatcggacgatccggcgacacctactatgctacatgggcaaaaggcaggttcacaattagtgctgatacttcaaagaacaccgcatacctgcagatgaatagtctgagggccgaagacactgctgtgtactattgctcccgcatcccttattttgggtggaacaatggagatatttgggggcagggaacactggtgactgtcagctcc

SEQ ID NO: 2 - protein, 119 aa, Artificial Sequence
  heavy chain of anti-cotinine scFv
EVQLVESGGGLVQPGGSLRLSCAASGHLRRRDWMNWVRQAPGKGLEWVAAIGRSGDTYYATWAKGRFTISADTSKNTAYLQMNSLRAEDTAVYYCSRIPYFGWNNGDIWGQGTLVTVSS

SEQ ID NO: 3 - DNA, 330 bp, Artificial Sequence
  light chain of anti-cotinine scFv
gacatccagatgacacagtctccatctagtctgagtgcatcagtgggcgatagagtcaccattacatgtcagtcaagccagagtccctactcaaacgagtggctgagctggtatcagcagaagcccggaaaagcccctaagctgctgatctacaggattagcacactggcttccggcgtgccttctcggttcagcggctccagatctgggactgactttactctgaccatctcctctctgcagccagaggatttcgcaacctactattgcgccggcgggtataattttggcctgttcctgtttggccaggggaccaaagtggaaattaag

SEQ ID NO: 4 - protein, 110 aa, Artificial Sequence
  light chain of anti-cotinine scFv
DIQMTQSPSSLSASVGDRVTITCQSSQSPYSNEWLSWYQQKPGKAPKLLIYRISTLASGVPSRFSGSRSGTDFTLTISSLQPEDFATYYCAGGYNFGLFLFGQGTKVEIK

SEQ ID NO: 5 - DNA, 1347 bp, Artificial Sequence
  heavy chain of cetuximab
caggtgcagctgaagcagagcggccccggactggtgcagccctcacagagcctgtccatcacttgcaccgtgagtggcttctcactgacaaactacggagtccactgggtgcgacagagccctggcaaggggctggagtggctgggcgtgatctggtccggagggaacactgactataatactcccttcaccagccggctgtccattaacaaggataactctaagagtcaggtgttctttaagatgaactctctgcagagtaatgacacagctatctactattgcgctcgcgcactgacttactatgattacgagttcgcatattggggacagggcacactggtcaccgtgagcgccgccagcaccaagggacccagcgtgtttccactggcccccagctccaaatcaaccagcggaggaacagcagccctgggatgtctggtgaaggactacttcccagaacccgtcacagtgtcctggaactctggggcactgacatctggagtccatacttttccagccgtgctgcagtctagtgggctgtacagcctgtcaagcgtggtcactgtcccctcctctagtctgggaacacagacttatatctgcaacgtgaatcacaagccaagtaataccaaggtcgacaaaagagtggagcccaagagctgtgataaaacccatacatgccccccttgtcctgcaccagaactgctggggggaccctccgtgttcctgtttccacccaagcctaaagacaccctgatgatttctaggactcccgaggtcacctgcgtggtcgtggacgtgagccacgaggatcctgaagtcaagttcaactggtacgtggatggcgtcgaagtgcataatgctaagacaaaacctcgggaggaacagtacaacagcacttatagagtcgtgtccgtcctgaccgtgctgcaccaggattggctgaacgggaaagagtataagtgcaaagtgagcaataaggccctgcccgctcctatcgagaaaaccatttccaaggccaaaggccagcctagggaaccacaggtgtacacactgcctccatcccgcgaggaaatgaccaagaaccaggtctctctgacatgtctggtgaaaggattctatccttcagacatcgctgtggagtgggaaagcaatggccagccagagaacaattacaagaccacaccccctgtgctggacagtgatggctcattctttctgtattctaagctgaccgtggataaaagtcgatggcagcaggggaatgtcttttcctgttctgtgatgcacgaagccctgcacaaccattacacccagaagagcctgagcctgtcccccggcaaa

SEQ ID NO: 6 - protein, 449 aa, Artificial Sequence
  heavy chain of cetuximab
QVQLKQSGPGLVQPSQSLSITCTVSGFSLTNYGVHWVRQSPGKGLEWLGVIWSGGNTDYNTPFTSRLSINKDNSKSQVFFKMNSLQSNDTAIYYCARALTYYDYEFAYWGQGTLVTVSAASTKGPSVFPLAPSSKSTSGGTAALGCLVKDYFPEPVTVSWNSGALTSGVHTFPAVLQSSGLYSLSSVVTVPSSSLGTQTYICNVNHKPSNTKVDKRVEPKSCDKTHTCPPCPAPELLGGPSVFLFPPKPKDTLMISRTPEVTCVVVDVSHEDPEVKFNWYVDGVEVHNAKTKPREEQYNSTYRVVSVLTVLHQDWLNGKEYKCKVSNKALPAPIEKTISKAKGQPREPQVYTLPPSREEMTKNQVSLTCLVKGFYPSDIAVEWESNGQPENNYKTTPPVLDSDGSFFLYSKLTVDKSRWQQGNVFSCSVMHEALHNHYTQKSLSLSPGK

SEQ ID NO: 7 - DNA, 642 bp, Artificial Sequence
  light chain of cetuximab
gatattctgctgactcagagccccgtgattctgtctgtcagccccggcgagcgggtgtctttcagttgcagagcatcacagagcatcggaacaaatattcactggtaccagcagaggactaacggctccccacgcctgctgatcaagtatgcttccgaatctatcagtgggattccctctcggttctcaggcagcgggtccggaacagactttactctgtctatcaatagtgtggagtcagaagacattgccgattactattgccagcagaacaataactggcctaccacattcggcgctgggaccaagctggagctgaaacgaacagtggccgctccaagtgtcttcatttttccccctagcgacgaacagctgaaatccgggaccgcctctgtggtctgtctgctgaataacttttaccctagagaggcaaaggtgcagtggaaagtcgataatgccctgcagagcggaaactcccaggagtctgtgactgaacaggacagtaaggattcaacctatagcctgagctccactctgaccctgtccaaagctgattacgaaaagcataaagtctatgcatgtgaggtcactcatcaggggctgtccagtccagtcaccaagtccttcaatcggggggaatgc

SEQ ID NO: 8 - protein, 214 aa, Artificial Sequence
  light chain of cetuximab
DILLTQSPVILSVSPGERVSFSCRASQSIGTNIHWYQQRTNGSPRLLIKYASESISGIPSRFSGSGSGTDFTLSINSVESEDIADYYCQQNNNWPTTFGAGTKLELKRTVAAPSVFIFPPSDEQLKSGTASVVCLLNNFYPREAKVQWKVDNALQSGNSQESVTEQDSKDSTYSLSSTLTLSKADYEKHKVYACEVTHQGLSSPVTKSFNRGEC

SEQ ID NO: 9 - protein, 214 aa, Artificial Sequence; identical to SEQ ID NO: 8
  light chain of tetravalent complex comprising bispecific cetuximab x anti-cotinine antibody

SEQ ID NO: 10 - protein, 715 aa, Artificial Sequence
  heavy chain of tetravalent complex comprising bispecific cetuximab x anti-cotinine antibody
QVQLKQSGPGLVQPSQSLSITCTVSGFSLTNYGVHWVRQSPGKGLEWLGVIWSGGNTDYNTPFTSRLSINKDNSKSQVFFKMNSLQSNDTAIYYCARALTYYDYEFAYWGQGTLVTVSAASTKGPSVFPLAPSSKSTSGGTAALGCLVKDYFPEPVTVSWNSGALTSGVHTFPAVLQSSGLYSLSSVVTVPSSSLGTQTYICNVNHKPSNTKVDKRVEPKSCDKTHTCPPCPAPELLGGPSVFLFPPKPKDTLMISRTPEVTCVVVDVSHEDPEVKFNWYVDGVEVHNAKTKPREEQYNSTYRVVSVLTVLHQDWLNGKEYKCKVSNKALPAPIEKTISKAKGQPREPQVYTLPPSREEMTKNQVSLTCLVKGFYPSDIAVEWESNGQPENNYKTTPPVLDSDGSFFLYSKLTVDKSRWQQGNVFSCSVMHEALHNHYTQKSLSLSPGKTSGGGGSGGGGSGGGGSEVQLVESGGGLVQPGGSLRLSCAASGHLRRRDWMNWVRQAPGKGLEWVAAIGRSGDTYYATWAKGRFTISADTSKNTAYLQMNSLRAEDTAVYYCSRIPYFGWNNGDIWGQGTLVTVSSGGGGSGGGGSGGGGSGGGGSDIQMTQSPSSLSASVGDRVTITCQSSQSPYSNEWLSWYQQKPGKAPKLLIYRISTLASGVPSRFSGSRSGTDFTLTISSLQPEDFATYYCAGGYNFGLFLFGQGTKVEIK